European Patent Application EP 4 317 424 A1, published February 7, 2024. Title: Vector for preparing a linear covalent closed DNA and a preparing method for a linear covalent closed DNA using thereof, and Preparing method for a parvovirus vector and a parvovirus vector producing cell. Applicant: KANEKA CORPORATION. The sequence listing filed with the application follows.

SEQUENCE LISTING (24 sequences)

SEQ ID NO: 1 - DNA, 1896 bp, Escherichia virus N15
  TelN
atgagcaaggtaaaaatcggtgagttgatcaacacgcttgtgaatgaggtagaggcaattgatgcctcagaccgcccacaaggcgacaaaacgaagagaattaaagccgcagccgcacggtataagaacgcgttatttaatgataaaagaaagttccgtgggaaaggattgcagaaaagaataaccgcgaatacttttaacgcctatatgagcagggcaagaaagcggtttgatgataaattacatcatagctttgataaaaatattaataaattatcggaaaagtatcctctttacagcgaagaattatcttcatggctttctatgcctacggctaatattcgccagcacatgtcatcgttacaatctaaattgaaagaaataatgccgcttgccgaagagttatcaaatgtaagaataggctctaaaggcagtgatgcaaaaatagcaagactaataaaaaaatatccagattggagttttgctcttagtgatttaaacagtgatgattggaaggagcgccgtgactatctttataagttattccaacaaggctctgcgttgttagaagaactacaccagctcaaggtcaaccatgaggttctgtaccatctgcagctaagccctgcggagcgtacatctatacagcaacgatgggccgatgttctgcgcgagaagaagcgtaatgttgtggttattgactacccaacatacatgcagtctatctatgatattttgaataatcctgcgactttatttagtttaaacactcgttctggaatggcacctttggcctttgctctggctgcggtatcagggcgaagaatgattgagataatgtttcagggtgaatttgccgtttcaggaaagtatacggttaatttctcagggcaagctaaaaaacgctctgaagataaaagcgtaaccagaacgatttatactttatgcgaagcaaaattattcgttgaattattaacagaattgcgttcttgctctgctgcatctgatttcgatgaggttgttaaaggatatggaaaggatgatacaaggtctgagaacggcaggataaatgctattttagcaaaagcatttaacccttgggttaaatcatttttcggcgatgaccgtcgtgtttataaagatagccgcgctatttacgctcgcatcgcttatgagatgttcttccgcgtcgatccacggtggaaaaacgtcgacgaggatgtgttcttcatggagattctcggacacgacgatgagaacacccagctgcactataagcagttcaagctggccaacttctccagaacctggcgacctgaagttggggatgaaaacaccaggctggtggctctgcagaaactggacgatgaaatgccaggctttgccagaggtgacgctggcgtccgtctccatgaaaccgttaagcagctggtggagcaggacccatcagcaaaaataaccaacagcactctccgggcctttaaatttagcccgacgatgattagccggtacctggagtttgccgctgatgcattggggcagttcgttggcgagaacgggcagtggcagctgaagatagagacacctgcaatcgtcctgcctgatgaagaatccgttgagaccatcgacgaaccggatgatgagtcccaagacgacgagctggatgaagatgaaattgagctcgacgagggtggcggcgatgaaccaaccgaagaggaagggccagaagaacatcagccaactgctctaaaacccgtcttcaagcctgcaaaaaataacggggacggaacgtacaagatagagtttgaatacgatggaaagcattatgcctggtccggccccgccgatagccctatggccgcaatgcgatccgcatgggaaacgtactacagctaa

SEQ ID NO: 2 - DNA, 56 bp, Artificial Sequence
  telRL
tatcagcacacaattgcccattatacgcgcgtataatggactattgtgtgctgata

SEQ ID NO: 3 - DNA, 1143 bp, Artificial Sequence
  AraC
gctaatcttatggataaaaatgctatggcatagcaaagtgtgacgccgtgcaaataatcaatgtggacttttctgccgtgattatagacacttttgttacgcgtttttgtcatggctttggtcccgctttgttacagaatgcttttaataagcggggttaccggtttggttagcgagaagagccagtaaaagacgcagtgacggcaatgtctgatgcaatatggacaattggtttcttctctgaatggcgggagtatgaaaagtatggctgaagcgcaaaatgatcccctgctgccgggatactcgtttaatgcccatctggtggcgggtttaacgccgattgaggccaacggttatctcgatttttttatcgaccgaccgctgggaatgaaaggttatattctcaatctcaccattcgcggtcagggggtggtgaaaaatcagggacgagaatttgtttgccgaccgggtgatattttgctgttcccgccaggagagattcatcactacggtcgtcatccggaggctcgcgaatggtatcaccagtgggtttactttcgtccgcgcgcctactggcatgaatggcttaactggccgtcaatatttgccaatacggggttctttcgcccggatgaagcgcaccagccgcatttcagcgacctgtttgggcaaatcattaacgccgggcaaggggaagggcgctattcggagctgctggcgataaatctgcttgagcaattgttactgcggcgcatggaagcgattaacgagtcgctccatccaccgatggataatcgggtacgcgaggcttgtcagtacatcagcgatcacctggcagacagcaattttgatatcgccagcgtcgcacagcatgtttgcttgtcgccgtcgcgtctgtcacatcttttccgccagcagttagggattagcgtcttaagctggcgcgaggaccaacgtatcagccaggcgaagctgcttttgagcaccacccggatgcctatcgccaccgtcggtcgcaatgttggttttgacgatcaactctatttctcgcgggtatttaaaaaatgcaccggggccagcccgagcgagttccgtgccggttgtgaagaaaaagtgaatgatgtagccgtcaagttgtcataa

SEQ ID NO: 4 - DNA, 55 bp, Artificial Sequence
  promoter
tacctgacgctttttatcgcaactctctactgtttctccatacccgtttttttgg

SEQ ID NO: 5 - DNA, 720 bp, Artificial Sequence
  Venus
atggtgagcaagggcgaggagctgttcaccggggtggtgcccatcctggtcgagctggacggcgacgtaaacggccacaagttcagcgtgtccggcgagggcgagggcgatgccacctacggcaagctgaccctgaagctgatctgcaccaccggcaagctgcccgtgccctggcccaccctcgtgaccaccctgggctacggcctgcagtgcttcgcccgctaccccgaccacatgaagcagcacgacttcttcaagtccgccatgcccgaaggctacgtccaggagcgcaccatcttcttcaaggacgacggcaactacaagacccgcgccgaggtgaagttcgagggcgacaccctggtgaaccgcatcgagctgaagggcatcgacttcaaggaggacggcaacatcctggggcacaagctggagtacaactacaacagccacaacgtctatatcaccgccgacaagcagaagaacggcatcaaggccaacttcaagatccgccacaacatcgaggacggcggcgtgcagctcgccgaccactaccagcagaacacccccatcggcgacggccccgtgctgctgcccgacaaccactacctgagctaccagtccgccctgagcaaagaccccaacgagaagcgcgatcacatggtcctgctggagttcgtgaccgccgccgggatcactctcggcatggacgagctgtacaagtaa

SEQ ID NO: 6 - DNA, 24 bp, Artificial Sequence
  TelN Fw
atgagcaaggtaaaaatcggtgag

SEQ ID NO: 7 - DNA, 23 bp, Artificial Sequence
  TelN Re
ttagctgtagtacgtttcccatg

SEQ ID NO: 8 - DNA, 27 bp, Artificial Sequence
  AraC Fw
gctaatcttatggataaaaatgctatg

SEQ ID NO: 9 - DNA, 24 bp, Artificial Sequence
  AraC Re
ttatgacaacttgacggctacatc

SEQ ID NO: 10 - DNA, 19 bp, Artificial Sequence
  Venus Fw
atggtgagcaagggcgagg

SEQ ID NO: 11 - DNA, 22 bp, Artificial Sequence
  Venus Re
ttacttgtacagctcgtccatg

SEQ ID NO: 12 - DNA, 1866 bp, Adeno associated virus
  Rep
atgccggggttttacgagattgtgattaaggtccccagcgaccttgacgagcatctgcccggcatttctgacagctttgtgaactgggtggccgagaaggaatgggagttgccgccagattctgacatggatctgaatctgattgagcaggcacccctgaccgtggccgagaagctgcagcgcgactttctgacggaatggcgccgtgtgagtaaggccccggaggcccttttctttgtgcaatttgagaagggagagagctacttccacatgcacgtgctcgtggaaaccaccggggtgaaatccatggttttgggacgtttcctgagtcagattcgcgaaaaactgattcagagaatttaccgcgggatcgagccgactttgccaaactggttcgcggtcacaaagaccagaaatggcgccggaggcgggaacaaggtggtggatgagtgctacatccccaattacttgctccccaaaacccagcctgagctccagtgggcgtggactaatatggaacagtatttaagcgcctgtttgaatctcacggagcgtaaacggttggtggcgcagcatctgacgcacgtgtcgcagacgcaggagcagaacaaagagaatcagaatcccaattctgatgcgccggtgatcagatcaaaaacttcagccaggtacatggagctggtcgggtggctcgtggacaaggggattacctcggagaagcagtggatccaggaggaccaggcctcatacatctccttcaatgcggcctccaactcgcggtcccaaatcaaggctgccttggacaatgcgggaaagattatgagcctgactaaaaccgcccccgactacctggtgggccagcagcccgtggaggacatttccagcaatcggatttataaaattttggaactaaacgggtacgatccccaatatgcggcttccgtctttctgggatgggccacgaaaaagttcggcaagaggaacaccatctggctgtttgggcctgcaactaccgggaagaccaacatcgcggaggccatagcccacactgtgcccttctacgggtgcgtaaactggaccaatgagaactttcccttcaacgactgtgtcgacaagatggtgatctggtgggaggaggggaagatgaccgccaaggtcgtggagtcggccaaagccattctcggaggaagcaaggtgcgcgtggaccagaaatgcaagtcctcggcccagatagacccgactcccgtgatcgtcacctccaacaccaacatgtgcgccgtgattgacgggaactcaacgaccttcgaacaccagcagccgttgcaagaccggatgttcaaatttgaactcacccgccgtctggatcatgactttgggaaggtcaccaagcaggaagtcaaagactttttccggtgggcaaaggatcacgtggttgaggtggagcatgaattctacgtcaaaaagggtggagccaagaaaagacccgcccccagtgacgcagatataagtgagcccaaacgggtgcgcgagtcagttgcgcagccatcgacgtcagacgcggaagcttcgatcaactacgcagacaggtaccaaaacaaatgttctcgtcacgtgggcatgaatctgatgctgtttccctgcagacaatgcgagagaatgaatcagaattcaaatatctgcttcactcacggacagaaagactgtttagagtgctttcccgtgtcagaatctcaacccgtttctgtcgtcaaaaaggcgtatcagaaactgtgctacattcatcatatcatgggaaaggtgccagacgcttgcactgcctgcgatctggtcaatgtggatttggatgactgcatctttgaacaataa

SEQ ID NO: 13 - DNA, 2208 bp, Adeno associated virus
  Cap
atggctgccgatggttatcttccagattggctcgaggacactctctctgaaggaataagacagtggtggaagctcaaacctggcccaccaccaccaaagcccgcagagcggcataaggacgacagcaggggtcttgtgcttcctgggtacaagtacctcggacccttcaacggactcgacaagggagagccggtcaacgaggcagacgccgcggccctcgagcacgacaaagcctacgaccggcagctcgacagcggagacaacccgtacctcaagtacaaccacgccgacgcggagtttcaggagcgccttaaagaagatacgtcttttgggggcaacctcggacgagcagtcttccaggcgaaaaagagggttcttgaacctctgggcctggttgaggaacctgttaagacggctccgggaaaaaagaggccggtagagcactctcctgtggagccagactcctcctcgggaaccggaaaggcgggccagcagcctgcaagaaaaagattgaattttggtcagactggagacgcagactcagtacctgacccccagcctctcggacagccaccagcagccccctctggtctgggaactaatacgatggctacaggcagtggcgcaccaatggcagacaataacgagggcgccgacggagtgggtaattcctcgggaaattggcattgcgattccacatggatgggcgacagagtcatcaccaccagcacccgaacctgggccctgcccacctacaacaaccacctctacaaacaaatttccagccaatcaggagcctcgaacgacaatcactactttggctacagcaccccttgggggtattttgacttcaacagattccactgccacttttcaccacgtgactggcaaagactcatcaacaacaactggggattccgacccaagagactcaacttcaagctctttaacattcaagtcaaagaggtcacgcagaatgacggtacgacgacgattgccaataaccttaccagcacggttcaggtgtttactgactcggagtaccagctcccgtacgtcctcggctcggcgcatcaaggatgcctcccgccgttcccagcagacgtcttcatggtgccacagtatggatacctcaccctgaacaacgggagtcaggcagtaggacgctcttcattttactgcctggagtactttccttctcagatgctgcgtaccggaaacaactttaccttcagctacacttttgaggacgttcctttccacagcagctacgctcacagccagagtctggaccgtctcatgaatcctctcatcgaccagtacctgtattacttgagcagaacaaacactccaagtggaaccaccacgcagtcaaggcttcagttttctcaggccggagcgagtgacattcgggaccagtctaggaactggcttcctggaccctgttaccgccagcagcgagtatcaaagacatctgcggataacaacaacagtgaatactcgtggactggagctaccaagtaccacctcaatggcagagactctctggtgaatccgggcccggccatggcaagccacaaggacgatgaagaaaagttttttcctcagagcggggttctcatctttgggaagcaaggctcagagaaaacaaatgtggacattgaaaaggtcatgattacagacgaagaggaaatcaggacaaccaatcccgtggctacggagcagtatggttctgtatctaccaacctccagagaggcaacagacaagcagctaccgcagatgtcaacacacaaggcgttcttccaggcatggtctggcaggacagagatgtgtaccttcaggggcccatctgggcaaagattccacacacggacggacattttcacccctctcccctcatgggtggattcggacttaaacaccctcctccacagattctcatcaagaacaccccggtacctgcgaatccttcgaccaccttcagtgcggcaaagtttgcttccttcatcacacagtactccacgggacaggtcagcgtggagatcgagtgggagctgcagaaggaaaacagcaaacgctggaatcccgaaattcagtacacttccaactacaacaagtctgttaatgtggactttactgtggacactaatggcgtgtattcagagcctcgccccattggcaccagatacctgactcgtaatctgtaa

SEQ ID NO: 14 - DNA, 5336 bp, Adenovirus
  E2A
ggtacccaactccatgcttaacagtccccaggtacagcccaccctgcgtcgcaaccaggaacagctctacagcttcctggagcgccactcgccctacttccgcagccacagtgcgcagattaggagcgccacttctttttgtcacttgaaaaacatgtaaaaataatgtactaggagacactttcaataaaggcaaatgtttttatttgtacactctcgggtgattatttaccccccacccttgccgtctgcgccgtttaaaaatcaaaggggttctgccgcgcatcgctatgcgccactggcagggacacgttgcgatactggtgtttagtgctccacttaaactcaggcacaaccatccgcggcagctcggtgaagttttcactccacaggctgcgcaccatcaccaacgcgtttagcaggtcgggcgccgatatcttgaagtcgcagttggggcctccgccctgcgcgcgcgagttgcgatacacagggttgcagcactggaacactatcagcgccgggtggtgcacgctggccagcacgctcttgtcggagatcagatccgcgtccaggtcctccgcgttgctcagggcgaacggagtcaactttggtagctgccttcccaaaaagggtgcatgcccaggctttgagttgcactcgcaccgtagtggcatcagaaggtgaccgtgcccggtctgggcgttaggatacagcgcctgcatgaaagccttgatctgcttaaaagccacctgagcctttgcgccttcagagaagaacatgccgcaagacttgccggaaaactgattggccggacaggccgcgtcatgcacgcagcaccttgcgtcggtgttggagatctgcaccacatttcggccccaccggttcttcacgatcttggccttgctagactgctccttcagcgcgcgctgcccgttttcgctcgtcacatccatttcaatcacgtgctccttatttatcataatgctcccgtgtagacacttaagctcgccttcgatctcagcgcagcggtgcagccacaacgcgcagcccgtgggctcgtggtgcttgtaggttacctctgcaaacgactgcaggtacgcctgcaggaatcgccccatcatcgtcacaaaggtcttgttgctggtgaaggtcagctgcaacccgcggtgctcctcgtttagccaggtcttgcatacggccgccagagcttccacttggtcaggcagtagcttgaagtttgcctttagatcgttatccacgtggtacttgtccatcaacgcgcgcgcagcctccatgcccttctcccacgcagacacgatcggcaggctcagcgggtttatcaccgtgctttcactttccgcttcactggactcttccttttcctcttgcgtccgcataccccgcgccactgggtcgtcttcattcagccgccgcaccgtgcgcttacctcccttgccgtgcttgattagcaccggtgggttgctgaaacccaccatttgtagcgccacatcttctctttcttcctcgctgtccacgatcacctctggggatggcgggcgctcgggcttgggagaggggcgcttctttttctttttggacgcaatggccaaatccgccgtcgaggtcgatggccgcgggctgggtgtgcgcggcaccagcgcatcttgtgacgagtcttcttcgtcctcggactcgagacgccgcctcagccgcttttttgggggcgcgcggggaggcggcggcgacggcgacggggacgacacgtcctccatggttggtggacgtcgcgccgcaccgcgtccgcgctcgggggtggtttcgcgctgctcctcttcccgactggccatttccttctcctataggcagaaaaagatcatggagtcagtcgagaaggaggacagcctaaccgccccctttgagttcgccaccaccgcctccaccgatgccgccaacgcgcctaccaccttccccgtcgaggcacccccgcttgaggaggaggaagtgattatcgagcaggacccaggttttgtaagcgaagacgacgaggatcgctcagtaccaacagaggataaaaagcaagaccaggacgacgcagaggcaaacgaggaacaagtcgggcggggggaccaaaggcatggcgactacctagatgtgggagacgacgtgctgttgaagcatctgcagcgccagtgcgccattatctgcgacgcgttgcaagagcgcagcgatgtgcccctcgccatagcggatgtcagccttgcctacgaacgccacctgttctcaccgcgcgtaccccccaaacgccaagaaaacggcacatgcgagcccaacccgcgcctcaacttctaccccgtatttgccgtgccagaggtgcttgccacctatcacatctttttccaaaactgcaagatacccctatcctgccgtgccaaccgcagccgagcggacaagcagctggccttgcggcagggcgctgtcatacctgatatcgcctcgctcgacgaagtgccaaaaatctttgagggtcttggacgcgacgagaaacgcgcggcaaacgctctgcaacaagaaaacagcgaaaatgaaagtcactgtggagtgctggtggaacttgagggtgacaacgcgcgcctagccgtgctgaaacgcagcatcgaggtcacccactttgcctacccggcacttaacctaccccccaaggttatgagcacagtcatgagcgagctgatcgtgcgccgtgcacgacccctggagagggatgcaaacttgcaagaacaaaccgaggagggcctacccgcagttggcgatgagcagctggcgcgctggcttgagacgcgcgagcctgccgacttggaggagcgacgcaagctaatgatggccgcagtgcttgttaccgtggagcttgagtgcatgcagcggttctttgctgacccggagatgcagcgcaagctagaggaaacgttgcactacacctttcgccagggctacgtgcgccaggcctgcaaaatttccaacgtggagctctgcaacctggtctcctaccttggaattttgcacgaaaaccgcctcgggcaaaacgtgcttcattccacgctcaagggcgaggcgcgccgcgactacgtccgcgactgcgtttacttatttctgtgctacacctggcaaacggccatgggcgtgtggcagcaatgcctggaggagcgcaacctaaaggagctgcagaagctgctaaagcaaaacttgaaggacctatggacggccttcaacgagcgctccgtggccgcgcacctggcggacattatcttccccgaacgcctgcttaaaaccctgcaacagggtctgccagacttcaccagtcaaagcatgttgcaaaactttaggaactttatcctagagcgttcaggaattctgcccgccacctgctgtgcgcttcctagcgactttgtgcccattaagtaccgtgaatgccctccgccgctttggggtcactgctaccttctgcagctagccaactaccttgcctaccactccgacatcatggaagacgtgagcggtgacggcctactggagtgtcactgtcgctgcaacctatgcaccccgcaccgctccctggtctgcaattcgcaactgcttagcgaaagtcaaattatcggtacctttgagctgcagggtccctcgcctgacgaaaagtccgcggctccggggttgaaactcactccggggctgtggacgtcggcttaccttcgcaaatttgtacctgaggactaccacgcccacgagattaggttctacgaagaccaatcccgcccgccaaatgcggagcttaccgcctgcgtcattacccagggccacatccttggccaattgcaagccatcaacaaagcccgccaagagtttctgctacgaaagggacggggggtttacctggacccccagtccggcgaggagctcaacccaatccccccgccgccgcagccctatcagcagccgcgggcccttgcttcccaggatggcacccaaaaagaagctgcagctgccgccgccgccacccacggacgaggaggaatactgggacagtcaggcagaggaggttttggacgaggaggaggagatgatggaagactgggacagcctagacgaagcttccgaggccgaagaggtgtcagacgaaacaccgtcaccctcggtcgcattcccctcgccggcgccccagaaattggcaaccgttcccagcatcgctacaacctccgctcctcaggcgccgccggcactgcctgttcgccgacccaaccgtagatgggacaccactggaaccagggccggtaagtctaagcagccgccgccgttagcccaagagcaacaacagcgccaaggctaccgctcgtggcgcgggcacaagaacgccatagttgcttgcttgcaagactgtgggggcaacatctccttcgcccgccgctttcttctctaccatcacggcgtggccttcccccgtaacatcctgcattactaccgtcatctctacagcccctactgcaccggcggcagcggcagcggcagcaacagcagcggtcacacagaagcaaaggcgaccggatagcaagactctgacaaagcccaagaaatccacagcggcggcagcagcaggaggaggagcgctgcgtctggcgcccaacgaacccgtatcgacccgcgagcttagaaataggatttttcccactctgtatgctatatttcaacaaagcaggggccaagaacaagagctgaaaataaaaaacaggtctctgcgctccctcacccgcagctgcctgtatcacaaaagcgaagatcagcttcggcgcacgctggaagacgcggaggctctcttcagcaaatactgcgcgctgactcttaaggactagtttcgcgccctttctcaaatttaagcgcgaaaactacgtcatctccagcggccacacccggcgccagcacctgtcgtcagcgccattatgagcaaggaaattcccacgccctacatgtggagttaccagccacaaatgggacttgcggctggagctgcccaagactactcaacccgaataaactacatgagcgcgggaccccacatgatatcccgggtcaacggaatccgcgcccaccgaaaccgaattctcctcgaacaggcggctattaccaccacacctcgtaataaccttaatccccgtagttggcccgctgccctggtgtaccaggaaagtcccgctcccaccactgtggtacttcccagagacgcccaggccgaagttcagatgactaactcaggggcgcagcttgcgggcggctttcgtcacagggtgcggtcg

SEQ ID NO: 15 - DNA, 3201 bp, Adenovirus
  E4
cccgggcgttttagggcggagtaacttgcatgtattgggaattgtagtttttttaaaatgggaagtgacgtatcgtgggaaaacggaagtgaagatttgaggaagttgtgggttttttggctttcgtttctgggcgtaggttcgcgtgcggttttctgggtgttttttgtggactttaaccgttacgtcattttttagtcctatatatactcgctctgtacttggccctttttacactgtgactgattgagctggtgccgtgtcgagtggtgttttttaataggtttttttactggtaaggctgactgttatggctgccgctgtggaagcgctgtatgttgttctggagcgggagggtgctattttgcctaggcaggagggtttttcaggtgtttatgtgtttttctctcctattaattttgttatacctcctatgggggctgtaatgttgtctctacgcctgcgggtatgtattcccccgggctatttcggtcgctttttagcactgaccgatgttaaccaacctgatgtgtttaccgagtcttacattatgactccggacatgaccgaggaactgtcggtggtgctttttaatcacggtgaccagtttttttacggtcacgccggcatggccgtagtccgtcttatgcttataagggttgtttttcctgttgtaagacaggcttctaatgtttaaatgtttttttttttgttattttattttgtgtttaatgcaggaacccgcagacatgtttgagagaaaaatggtgtctttttctgtggtggttccggaacttacctgcctttatctgcatgagcatgactacgatgtgcttgcttttttgcgcgaggctttgcctgattttttgagcagcaccttgcattttatatcgccgcccatgcaacaagcttacataggggctacgctggttagcatagctccgagtatgcgtgtcataatcagtgtgggttcttttgtcatggttcctggcggggaagtggccgcgctggtccgtgcagacctgcacgattatgttcagctggccctgcgaagggacctacgggatcgcggtatttttgttaatgttccgcttttgaatcttatacaggtctgtgaggaacctgaatttttgcaatcatgattcgctgcttgaggctgaaggtggagggcgctctggagcagatttttacaatggccggacttaatattcgggatttgcttagagacatattgataaggtggcgagatgaaaattatttgggcatggttgaaggtgctggaatgtttatagaggagattcaccctgaagggtttagcctttacgtccacttggacgtgagggcagtttgccttttggaagccattgtgcaacatcttacaaatgccattatctgttctttggctgtagagtttgaccacgccaccggaggggagcgcgttcacttaatagatcttcattttgaggttttggataatcttttggaataaaaaaaaaaaaacatggttcttccagctcttcccgctcctcccgtgtgtgactcgcagaacgaatgtgtaggttggctgggtgtggcttattctgcggtggtggatgttatcagggcagcggcgcatgaaggagtttacatagaacccgaagccagggggcgcctggatgctttgagagagtggatatactacaactactacacagagcgagctaagcgacgagaccggagacgcagatctgtttgtcacgcccgcacctggttttgcttcaggaaatatgactacgtccggcgttccatttggcatgacactacgaccaacacgatctcggttgtctcggcgcactccgtacagtagggatcgcctacctccttttgagacagagacccgcgctaccatactggaggatcatccgctgctgcccgaatgtaacactttgacaatgcacaacgtgagttacgtgcgaggtcttccctgcagtgtgggatttacgctgattcaggaatgggttgttccctgggatatggttctgacgcgggaggagcttgtaatcctgaggaagtgtatgcacgtgtgcctgtgttgtgccaacattgatatcatgacgagcatgatgatccatggttacgagtcctgggctctccactgtcattgttccagtcccggttccctgcagtgcatagccggcgggcaggttttggccagctggtttaggatggtggtggatggcgccatgtttaatcagaggtttatatggtaccgggaggtggtgaattacaacatgccaaaagaggtaatgtttatgtccagcgtgtttatgaggggtcgccacttaatctacctgcgcttgtggtatgatggccacgtgggttctgtggtccccgccatgagctttggatacagcgccttgcactgtgggattttgaacaatattgtggtgctgtgctgcagttactgtgctgatttaagtgagatcagggtgcgctgctgtgcccggaggacaaggcgtctcatgctgcgggcggtgcgaatcatcgctgaggagaccactgccatgttgtattcctgcaggacggagcggcggcggcagcagtttattcgcgcgctgctgcagcaccaccgccctatcctgatgcacgattatgactctacccccatgtaggcgtggacttccccttcgccgcccgttgagcaaccgcaagttggacagcagcctgtggctcagcagctggacagcgacatgaacttaagcgagctgcccggggagtttattaatatcactgatgagcgtttggctcgacaggaaaccgtgtggaatataacacctaagaatatgtctgttacccatgatatgatgctttttaaggccagccggggagaaaggactgtgtactctgtgtgttgggagggaggtggcaggttgaatactagggttctgtgagtttgattaaggtacggtgatcaatataagctatgtggtggtggggctatactactgaatgaaaaatgacttgaaattttctgcaattgaaaaataaacacgttgaaacataacatgcaacaggttcacgattctttattcctgggcaatgtaggagaaggtgtaagagttggtagcaaaagtttcagtggtgtattttccactttcccaggaccatgtaaaagacatagagtaagtgcttacctcgctagtttctgtggattcactagaa

SEQ ID NO: 16 - DNA, 743 bp, Adenovirus
  VA
tcgatgtaggatgttgcccctcctgacgcggtaggagaaggggagggtgccctgcatgtctgccgctgctcttgctcttgccgctgctgaggaggggggcgcatctgccgcagcaccggatgcatctgggaaaagcaaaaaaggggctcgtccctgtttccggaggaatttgcaagcggggtcttgcatgacggggaggcaaacccccgttcgccgcagtccggccggcccgagactcgaaccgggggtcctgcgactcaacccttggaaaataaccctccggctacagggagcgagccacttaatgctttcgctttccagcctaaccgcttacgccgcgcgcggccagtggccaaaaaagctagcgcagcagccgccgcgcctggaaggaagccaaaaggagcgctcccccgttgtctgacgtcgcacacctgggttcgacacgcgggcggtaaccgcatggatcacggcggacggccggatccggggttcgaaccccggtcgtccgccatgatacccttgcgaatttatccaccagaccacggaagagtgcccgcttacaggctctccttttgcacggtctagagcgtcaacgactgcgcacgcctcaccggccagagcgtcccgaccatggagcactttttgccgctgcgcaacatctggaaccgcgtccgcgactttccgcgcgcctccaccaccgccgccggcatcacctggatgtccaggtacatctacggattacg

SEQ ID NO: 17 - DNA, 43 bp, Artificial Sequence
  Helper Fw
gtacatcaagtgtatcatatgggtacccaactccatgcttaac

SEQ ID NO: 18 - DNA, 45 bp, Artificial Sequence
  Helper Re
agggggcgtacttggcatatggtcgacgtaatccgtagatgtacc

SEQ ID NO: 19 - DNA, 19 bp, Artificial Sequence
  Venus Fw
cacaacgtctatatcaccg

SEQ ID NO: 20 - DNA, 16 bp, Artificial Sequence
  Venus Re
tgtgatcgcgcttctc

SEQ ID NO: 21 - DNA, 16 bp, Artificial Sequence
  Amp Fw
atcccgtattgacgcc

SEQ ID NO: 22 - DNA, 16 bp, Artificial Sequence
  Amp Re
cgctcgtcgtttggta

SEQ ID NO: 23 - DNA, 1292 bp, Artificial Sequence
  LacI
tcactgcccgctttccagtcgggaaacctgtcgtgccagctgcattaatgaatcggccaacgcgcggggagaggcggtttgcgtattgggcgccagggtggtttttcttttcaccagtgagacgggcaacagctgattgcccttcaccgcctggccctgagagagttgcagcaagcggtccacgctggtttgccccagcaggcgaaaatcctgtttgatggtggttaacggcgggatataacatgagctgtcttcggtatcgtcgtatcccactaccgagatatccgcaccaacgcgcagcccggactcggtaatggcgcgcattgcgcccagcgccatctgatcgttggcaaccagcatcgcagtgggaacgatgccctcattcagcatttgcatggtttgttgaaaaccggacatggcactccagtcgccttcccgttccgctatcggctgaatttgattgcgagtgagatatttatgccagccagccagacgcagacgcgccgagacagaacttaatgggcccgctaacagcgcgatttgctggtgacccaatgcgaccagatgctccacgcccagtcgcgtaccgtcttcatgggagaaaataatactgttgatgggtgtctggtcagagacatcaagaaataacgccggaacattagtgcaggcagcttccacagcaatggcatcctggtcatccagcggatagttaatgatcagcccactgacgcgttgcgcgagaagattgtgcaccgccgctttacaggcttcgacgccgcttcgttctaccatcgacaccaccacgctggcacccagttgatcggcgcgagatttaatcgccgcgacaatttgcgacggcgcgtgcagggccagactggaggtggcaacgccaatcagcaacgactgtttgcccgccagttgttgtgccacgcggttgggaatgtaattcagctccgccatcgccgcttccactttttcccgcgttttcgcagaaacgtggctggcctggttcaccacgcgggaaacggtctgataagagacaccggcatactctgcgacatcgtataacgttactggtttcacattcaccaccctgaattgactctcttccgggcgctatcatgccataccgcgaaaggttttgcgccattcgatggtgtccgggatctcgacgctctcccttatgcgactcctgcattaggaagcagcccagtagtaggttgaggccgttgagcaccgccgccgcaaggaatggtgcatgcaaggagatggcgcccaacagtcccccggcc

SEQ ID NO: 24 - DNA, 35 bp, Artificial Sequence
  promoter
ttgacaattaatcatcggctcgtataatgtgtgga